European Patent Application EP 4 491 729 A1, published January 15, 2025. Title: Ｅｖａ１タンパク質に結合する、ヒト化抗体又はその機能的断片、抗体薬物複合体及びキメラ抗原受容体. Applicant: CURED Inc. The sequence listing filed with the application follows.

SEQUENCE LISTING (66 sequences)

SEQ ID NO: 1 - protein, 5 aa, synthetic construct
  REGION 1..5: note = CDR1 of Light Chain (Humanized B2E5-48)
SSVGY

SEQ ID NO: 2 - skipped

SEQ ID NO: 3 - protein, 9 aa, synthetic construct
  REGION 1..9: note = CDR3 of Light Chain (Humanized B2E5-48)
QQWSSNPPT

SEQ ID NO: 4 - protein, 8 aa, synthetic construct
  REGION 1..8: note = CDR1 of Heavy Chain (Humanized B2E5-48)
GYTFTNYW

SEQ ID NO: 5 - protein, 8 aa, synthetic construct
  REGION 1..8: note = CDR2 of Heavy Chain (Humanized B2E5-48)
INPTNGGT

SEQ ID NO: 6 - protein, 9 aa, synthetic construct
  REGION 1..9: note = CDR3 of Heavy Chain (Humanized B2E5-48)
TIYTTALDY

SEQ ID NO: 7 - protein, 106 aa, synthetic construct
  REGION 1..106: note = Variable Region of Light Chain 2 (Humanized B2E5-48)
EIVLTQSPATLSLSPGERATLSCRASSSVGYMYWYQQKPGQAPRPLIYVTSNRATGIPARFSGSGSGTDYTLTISSLEPEDFAVYYCQQWSSNPPTFGQGTKLEIK

SEQ ID NO: 8 - protein, 106 aa, synthetic construct
  REGION 1..106: note = Variable Region of Light Chain 4 (Humanized B2E5-48)
DIQLTQSPSFLSASVGDRVTITCRASSSVGYMYWYQQKPGKAPKPLIYVTSNLASGVPSRFSGSGSGTEYTLTISSLQPEDFATYYCQQWSSNPPTFGQGTKLEIK

SEQ ID NO: 9 - protein, 106 aa, synthetic construct
  REGION 1..106: note = Variable Region of Light Chain 1 (Humanized B2E5-48)
QIVLTQSPATLSLSPGERATLSCRASSSVGYMYWYQQKPGQAPRPLIYVTSNLASGIPARFSGSGSGTDYTLTISSLEPEDFAVYYCQQWSSNPPTFGQGTKLEIK

SEQ ID NO: 10 - protein, 106 aa, synthetic construct
  REGION 1..106: note = Variable Region of Light Chain 3 (Humanized B2E5-48)
QIQLTQSPSFLSASVGDRVTITCRASSSVGYMYWYQQKPGKAPKPLIYVTSNLASGVPSRFSGSGSGTEYTLTISSLQPEDFATYYCQQWSSNPPTFGQGTKLEIK

SEQ ID NO: 11 - DNA, 318 bp, synthetic construct
  misc_feature 1..318: note = Variable Region of Light Chain 2 (Humanized B2E5-48) cDNA
  source 1..318: mol_type = other DNA
gagatcgtgctgacccagagccccgccacactgtctctgagccccggcgagagagccacactgagctgcagagccagctcctccgtgggctacatgtactggtaccagcaaaagcccggacaagcccccagacctctgatttacgtgaccagcaacagagccaccggcatccccgccagatttagcggaagcggcagcggcaccgactacacactgaccatctcctctctggagccagaggacttcgccgtgtactactgccagcagtggagctccaaccctcccaccttcggccaaggcaccaagctcgagatcaag

SEQ ID NO: 12 - DNA, 318 bp, synthetic construct
  misc_feature 1..318: note = Variable Region of Light Chain 4 (Humanized B2E5-48) cDNA
  source 1..318: mol_type = other DNA
gacatccagctgacccagtccccttcctttctgagcgcttccgtgggcgacagagtgaccatcacatgcagagccagcagcagcgtgggctacatgtactggtaccagcagaagcccggaaaggcccccaagcctctgatctacgtgaccagcaatctggccagcggcgtgcccagcagatttagcggctccggcagcggcacagagtatacactgaccatcagctctctgcagccagaggacttcgccacctactactgccagcagtggagctccaacccccccacctttggccaaggcaccaagctcgagatcaag

SEQ ID NO: 13 - protein, 116 aa, synthetic construct
  REGION 1..116: note = Variable Region of Heavy Chain 2 (Humanized B2E5-48)
QVQLVQSGAEVKKPGASVKVSCKASGYTFTNYWMHWVRQAPGQGLEWMGEINPTNGGTDYNEKFQGRVTMTVDKSTSTAYMELSSLRSEDTAVYYCTIYTTALDYWGQGTLVTVSS

SEQ ID NO: 14 - protein, 116 aa, synthetic construct
  REGION 1..116: note = Variable Region of Heavy Chain 4 (Humanized B2E5-48)
QVQLVQSGSELKKPGASVKVSCKASGYTFTNYWMHWVRQAPGQGLEWMGEINPTNGGTDYNEGFTGRFVFSVDKSVSTAYLQISSLKAEDTAVYYCTIYTTALDYWGQGTLVTVSS

SEQ ID NO: 15 - protein, 116 aa, synthetic construct
  REGION 1..116: note = Variable Region of Heavy Chain 1 (Humanized B2E5-48)
QVQLVQSGAEVKKPGASVKVSCKASGYTFTNYWMHWVRQAPGQGLEWIGEINPTNGGTDYNEKFQGRVTLTVDKSSSTAYMELSSLRSEDTAVYYCTIYTTALDYWGQGTLVTVSS

SEQ ID NO: 16 - protein, 116 aa, synthetic construct
  REGION 1..116: note = Variable Region of Heavy Chain 3 (Humanized B2E5-48)
QVQLVQSGSELKKPGASVKVSCKASGYTFTNYWMHWVRQAPGQGLEWIGEINPTNGGTDYNEGFTGRFVLSVDKSSSTAYLQISSLKAEDTAVYYCTIYTTALDYWGQGTLVTVSS

SEQ ID NO: 17 - DNA, 348 bp, synthetic construct
  misc_feature 1..348: note = Variable Region of Heavy Chain 2 (Humanized B2E5-48) cDNA
  source 1..348: mol_type = other DNA
caagtgcagctggtgcagagcggagccgaagtgaagaaacccggagcctccgtgaaggtgagctgcaaggccagcggatacaccttcaccaactactggatgcactgggtgagacaagcccccggccaaggactggagtggatgggcgagatcaaccccaccaacggcggcaccgactacaatgagaagttccaaggaagagtgaccatgacagtggacaagagcaccagcaccgcctacatggagctgagctctctgaggtccgaggacaccgccgtgtactactgcaccatctacaccaccgctctggattactggggccaaggcacactggtgaccgtctcgagc

SEQ ID NO: 18 - DNA, 348 bp, synthetic construct
  misc_feature 1..348: note = Variable Region of Heavy Chain 3 (Humanized B2E5-48) cDNA
  source 1..348: mol_type = other DNA
caagtgcagctggtgcagtccggcagcgagctgaagaagcccggagccagcgtgaaggtgagctgcaaggccagcggctacaccttcaccaactactggatgcactgggtgagacaagcccccggccaaggactggagtggattggcgagatcaaccctaccaacggcggcaccgactacaatgagggcttcaccggaagattcgtgctgtccgtggacaaatccagctccacagcctacctccagatcagctctctgaaggccgaggataccgccgtgtactactgcaccatctacaccaccgctctggattactggggccaaggcacactggtgacagtctcgagc

SEQ ID NO: 19 - DNA, 384 bp, Mus musculus
  source 1..384: mol_type = other DNA
  CDS 1..384: note = Signal peptide and Variable Region of Light Chain (B2E5-48)
atggattttcaagtgcagattttcagcttcctgctaatgagtgcctcagtcataatgtccaggggacaaattgttctcacccagtctccagcactcatgtctgcatctccaggggagagggtcaccttgacctgcagtgccagctcaagtgtaggttacatgtactggtaccagcagaagccaggatcctcccccaaaccctggatttatgtcacatccaacctggcttctggagtccctgctcgcttcagtggcagtgggtctgggacctcttactctctcacaatcagcagcatggaggctgaagatgctgccacttattactgccagcagtggagtagtaacccacctacgttcggtgctgggaccaagctggagctgaaa

SEQ ID NO: 20 - protein, 128 aa, Mus musculus
MDFQVQIFSFLLMSASVIMSRGQIVLTQSPALMSASPGERVTLTCSASSSVGYMYWYQQKPGSSPKPWIYVTSNLASGVPARFSGSGSGTSYSLTISSMEAEDAATYYCQQWSSNPPTFGAGTKLELK

SEQ ID NO: 21 - protein, 106 aa, Mus musculus
  SITE 1..106: note = Variable Region of Light Chain (B2E5-48)
QIVLTQSPALMSASPGERVTLTCSASSSVGYMYWYQQKPGSSPKPWIYVTSNLASGVPARFSGSGSGTSYSLTISSMEAEDAATYYCQQWSSNPPTFGAGTKLELK

SEQ ID NO: 22 - protein, 10 aa, Mus musculus
  SITE 1..10: note = CDR1 of Light Chain (B2E5-48)
SASSSVGYMY

SEQ ID NO: 23 - protein, 7 aa, Mus musculus
  SITE 1..7: note = CDR2 of Light Chain (B2E5-48)
VTSNLAS

SEQ ID NO: 24 - protein, 9 aa, Mus musculus
  SITE 1..9: note = CDR3 of Light Chain (B2E5-48)
QQWSSNPPT

SEQ ID NO: 25 - DNA, 405 bp, Mus musculus
  source 1..405: mol_type = other DNA
  CDS 1..405: note = Signal peptide and Variable Region of Heavy Chain (B2E5-48)
atgggatggagctacatcattttctttttggtagcaacagctacaggtgtccactcccaggtccaactccagcagcctggggctgaactggtgaagcctggggcttcagtgaagttgtcctgcaaggcttctggctacaccttcaccaactactggatgcactgggtgaagctgaggcctggacaaggctttgagtggattggagagattaatcctaccaatggtggtactgactacaatgagaagttcaagagaaaggccacactgactgtagacaaatcctccagcacagcctacatgcaactcagcagcctgacatctgaggactctgcggtctattactgcacaatatatactacggctcttgactactggggccaaggcaccactctcacagtctcctca

SEQ ID NO: 26 - protein, 135 aa, Mus musculus
MGWSYIIFFLVATATGVHSQVQLQQPGAELVKPGASVKLSCKASGYTFTNYWMHWVKLRPGQGFEWIGEINPTNGGTDYNEKFKRKATLTVDKSSSTAYMQLSSLTSEDSAVYYCTIYTTALDYWGQGTTLTVSS

SEQ ID NO: 27 - protein, 116 aa, Mus musculus
  SITE 1..116: note = Variable Region of Heavy Chain (B2E5-48)
QVQLQQPGAELVKPGASVKLSCKASGYTFTNYWMHWVKLRPGQGFEWIGEINPTNGGTDYNEKFKRKATLTVDKSSSTAYMQLSSLTSEDSAVYYCTIYTTALDYWGQGTTLTVSS

SEQ ID NO: 28 - protein, 7 aa, Mus musculus
  SITE 1..7: note = CDR1 of Heavy Chain (B2E5-48)
GYTFTNY

SEQ ID NO: 29 - protein, 6 aa, Mus musculus
  SITE 1..6: note = CDR2 of Heavy Chain (B2E5-48)
NPTNGG

SEQ ID NO: 30 - protein, 7 aa, Mus musculus
  SITE 1..7: note = CDR3 of Heavy Chain (B2E5-48)
YTTALDY

SEQ ID NO: 31 - DNA, 381 bp, Mus musculus
  source 1..381: mol_type = other DNA
  CDS 1..381: note = Signal peptide and Variable Region of Light Chain (C3)
atgaagtcacagacccaggtcttcgtatttctactgctctgtgtgtctggtgctcatgggagtattgtgatgacccagactcccaaattcctgcttgtatcagcaggagacagggttaccataacctgcaaggccagtcagagtgtgagtaatgatgtagcttggtaccaacagaagccagggcagtctcctaaactgctgatatactatgcatccaatcgctacactggagtccctgatcgcttcactggcagtggatatgggacggatttcactttcaccatcagcactgtgcaggctgaagacctggcagtttatttctgtcagcaggattatagctctccgtggacgttcggtggaggcaccaagctggaaatcaaa

SEQ ID NO: 32 - protein, 127 aa, Mus musculus
MKSQTQVFVFLLLCVSGAHGSIVMTQTPKFLLVSAGDRVTITCKASQSVSNDVAWYQQKPGQSPKLLIYYASNRYTGVPDRFTGSGYGTDFTFTISTVQAEDLAVYFCQQDYSSPWTFGGGTKLEIK

SEQ ID NO: 33 - protein, 107 aa, Mus musculus
  SITE 1..107: note = Variable Region of Light Chain (C3)
SIVMTQTPKFLLVSAGDRVTITCKASQSVSNDVAWYQQKPGQSPKLLIYYASNRFTGVPDRFTGSGYGTDFTFTISTVQAEDLAVYFCQQDYSSPWTFGGGTKLEIK

SEQ ID NO: 34 - protein, 11 aa, Mus musculus
  SITE 1..11: note = CDR1 of Light Chain (C3)
KASQSVSNDVA

SEQ ID NO: 35 - protein, 7 aa, Mus musculus
  SITE 1..7: note = CDR2 of Light Chain (C3)
YASNRFT

SEQ ID NO: 36 - protein, 9 aa, Mus musculus
  SITE 1..9: note = CDR3 of Light Chain (C3)
QQDYSSPWT

SEQ ID NO: 37 - DNA, 402 bp, Mus musculus
  source 1..402: mol_type = other DNA
  CDS 1..402: note = Signal peptide and Variable Region of Heavy Chain (C3)
atgaatttcgggctcagcttgattttccttgtccttgttttaaaaggtgtcctgtgtgaagtgaaactggtggagtctgggggaggtttagtgcagcctggagggtccctgaaactctcctgtgcagcctctggattcactttcagtagctataccatgtcttgggttcgccagactccagagaagaggctggagtgggtcgcatacattactactggtgctggtaggacctactatccagacactgtaaagggccgattcaccatctccagagacaatgccaagaacaccctgtacctgcaaatgagtagtctgaagtctgaggacacggccatgtattactgtgcaagacatcggggggactactggggtcaaggaacctcagtcaccgtctcctcagcc

SEQ ID NO: 38 - protein, 134 aa, Mus musculus
MNFGLSLIFLVLVLKGVLCEVKLVESGGGLVQPGGSLKLSCAASGFTFSSYTMSWVRQTPEKRLEWVAYITTGAGRTYYPDTVKGRFTISRDNAKNTLYLQMSSLKSEDTAMYYCARHRGDYWGQGTSVTVSSA

SEQ ID NO: 39 - protein, 115 aa, Mus musculus
  SITE 1..115: note = Variable Region of Heavy Chain (C3)
EVKLVESGGGLVQPGGSLKLSCAASGFTFSSYTMSWVRQTPEKRLEWVAYITTGAGRTYYPDTVKGRFTISRDNAKNTLYLQMSSLKSEDTAMYYCARHRGDYWGQGTSVTVSSA

SEQ ID NO: 40 - protein, 7 aa, Mus musculus
  SITE 1..7: note = CDR1 of Heavy Chain (C3)
GFTFSSY

SEQ ID NO: 41 - protein, 6 aa, Mus musculus
  SITE 1..6: note = CDR2 of Heavy Chain (C3)
TTGAGR

SEQ ID NO: 42 - protein, 5 aa, Mus musculus
  SITE 1..5: note = CDR3 of Heavy Chain (C3)
HRGDY

SEQ ID NO: 43 - DNA, 324 bp, Mus musculus
  source 1..324: mol_type = other DNA
  CDS 1..324: note = Variable Region of Light Chain (A5D11-10)
gatatccagatgacacagactacatcttccctgtctgcctctctgggagacagagtcaccatcagttgcagggcaagtcaggacattagcaattatttaaactggtatcagcagaaaccagatggaactgttaaactccttatctactacacatcaagattacactcaggagtcccatcaaggttcagtggcagtgggtctcgaatagattattctctcaccattagcaacctggagcaagaagattttgccacttacttttgccaacagagtgatacgcttcctccgtggacgttcggtggaggcaccaagctggaaatcaaa

SEQ ID NO: 44 - protein, 108 aa, Mus musculus
DIQMTQTTSSLSASLGDRVTISCRASQDISNYLNWYQQKPDGTVKLLIYYTSRLHSGVPSRFSGSGSRIDYSLTISNLEQEDFATYFCQQSDTLPPWTFGGGTKLEIK

SEQ ID NO: 45 - protein, 11 aa, Mus musculus
  SITE 1..11: note = CDR1 of Light Chain (A5D11-10)
RASQDISNYLN

SEQ ID NO: 46 - protein, 7 aa, Mus musculus
  SITE 1..7: note = CDR2 of Light Chain (A5D11-10)
YTSRLHS

SEQ ID NO: 47 - protein, 10 aa, Mus musculus
  SITE 1..10: note = CDR3 of Light Chain (A5D11-10)
QQSDTLPPWT

SEQ ID NO: 48 - DNA, 357 bp, Mus musculus
  source 1..357: mol_type = other DNA
  CDS 1..357: note = Variable Region of Heavy Chain (A5D11-10)
gaggtgcagctgaaggagtcaggacctggcctagtgcagccctcacagagcctgtccatcacctgcacagtctctggtttctcattaactaggtatggtgtacactgggttcgccagtctccaggaaagggtctggagtggctgggagtgatatggagtggtggaagcacagactataatgcagctttcatatccagactgagcatcagcaaggacaattccaagagccaagttttctttaaaatgaacagtctgcaagctaatgacacagccatatattactgtgccagaaatggttacgacgggggctatgctatggactactggggtcaaggaacctcagtcaccgtctcctca

SEQ ID NO: 49 - protein, 119 aa, Mus musculus
EVQLKESGPGLVQPSQSLSITCTVSGFSLTRYGVHWVRQSPGKGLEWLGVIWSGGSTDYNAAFISRLSISKDNSKSQVFFKMNSLQANDTAIYYCARNGYDGGYAMDYWGQGTSVTVSS

SEQ ID NO: 50 - protein, 7 aa, Mus musculus
  SITE 1..7: note = CDR1 of Heavy Chain (A5D11-10)
GFSLTRY

SEQ ID NO: 51 - protein, 5 aa, Mus musculus
  SITE 1..5: note = CDR2 of Heavy Chain (A5D11-10)
WSGGS

SEQ ID NO: 52 - protein, 11 aa, Mus musculus
  SITE 1..11: note = CDR3 of Heavy Chain (A5D11-10)
NGYDGGYAMDY

SEQ ID NO: 53 - DNA, 648 bp, Homo sapiens
  source 1..648: mol_type = other DNA
  CDS 1..648: note = hEva1; protein_id = 54; translation = MYGKSSTRAVLLLLGIQLTALWPIAAVEIYTSRVLEAVNGTDARLKCTFSSFAPVGDALTVTWNFRPLDGGPEQFVFYYHIDPFQPMSGRFKDRVSWDGNPERYDASILLWKLQFDDNGTYTCQVKNPPDVDGVIGEIRLSVVHTVRFSEIHFLALAIGSACALMIIIVIVVVLFQHYRKKRWAERAHKVVEIKSKEEERLNQEKKVSVYLEDTD
atgtatggcaagagctctactcgtgcggtgcttcttctccttggcatacagctcacagctctttggcctatagcagctgtggaaatttatacctcccgggtgctggaggctgttaatgggacagatgctcggttaaaatgcactttctccagctttgcccctgtgggtgatgctctaacagtgacctggaattttcgtcctctagacgggggacctgagcagtttgtattctactaccacatagatcccttccaacccatgagtgggcggtttaaggaccgggtgtcttgggatgggaatcctgagcggtacgatgcctccatccttctctggaaactgcagttcgacgacaatgggacatacacctgccaggtgaagaacccacctgatgttgatggggtgataggggagatccggctcagcgtcgtgcacactgtacgcttctctgagatccacttcctggctctggccattggctctgcctgtgcactgatgatcataatagtaattgtagtggtcctcttccagcattaccggaaaaagcgatgggccgaaagagctcataaagtggtggagataaaatcaaaagaagaggaaaggctcaaccaagagaaaaaggtctctgtttatttagaagacacagactaa

SEQ ID NO: 54 - protein, 215 aa, Homo sapiens
MYGKSSTRAVLLLLGIQLTALWPIAAVEIYTSRVLEAVNGTDARLKCTFSSFAPVGDALTVTWNFRPLDGGPEQFVFYYHIDPFQPMSGRFKDRVSWDGNPERYDASILLWKLQFDDNGTYTCQVKNPPDVDGVIGEIRLSVVHTVRFSEIHFLALAIGSACALMIIIVIVVVLFQHYRKKRWAERAHKVVEIKSKEEERLNQEKKVSVYLEDTD

SEQ ID NO: 55 - DNA, 648 bp, Mus musculus
  source 1..648: mol_type = other DNA
  CDS 1..648: note = mEva1; protein_id = 56; translation = MYGKSPALVLPLLLSLQLTALCPTEAVEIYTSGALEAVNGTDVRLKCTFSSFAPVGDALTVTWNFRPRDGGREQFVFYYHMDPFRPMSGRFKDRVVWDGNPERYDVSILLWKLQFDDNGTYTCQVKNPPDVDGLVGTIRLSVVHTVPFSEIYFLAVAIGSACALMIIVVIVVVLFQHFRKKRWADSADKAEGTKSKEEEKLNQGNKVSVFVEDTD
atgtatggcaagagccccgcgcttgtgcttccacttctcctgagtttacagctcacagccctttgtcctacagaagctgtggaaatttacacctccggggccctggaggcagtcaacgggacagatgttcggttaaaatgcactttctccagctttgcccctgtgggagatgcgctaactgtgacgtggaatttccgacctcgagatgggggtcgtgagcagtttgtattctactaccacatggaccccttcaggcccatgagcggacggttcaaagaccgggtggtctgggacggaaaccccgagcgatatgacgtctccatcttgctctggaagctgcagtttgacgacaatgggacatacacctgccaggtgaagaatccacctgatgttgatggtctggttgggacgatccggctcagcgttgtgcacactgtgcccttctctgagatctacttcctggccgtggccattggctctgcgtgcgcactgatgatcatcgtagtgatcgtggtagtcctcttccagcacttccggaaaaagcgatgggcggacagtgctgataaagccgaggggacaaaatcaaaagaagaggaaaaactcaaccaaggaaacaaggtctctgtttttgtggaagatacagactaa

SEQ ID NO: 56 - protein, 215 aa, Mus musculus
MYGKSPALVLPLLLSLQLTALCPTEAVEIYTSGALEAVNGTDVRLKCTFSSFAPVGDALTVTWNFRPRDGGREQFVFYYHMDPFRPMSGRFKDRVVWDGNPERYDVSILLWKLQFDDNGTYTCQVKNPPDVDGLVGTIRLSVVHTVPFSEIYFLAVAIGSACALMIIVVIVVVLFQHFRKKRWADSADKAEGTKSKEEEKLNQGNKVSVFVEDTD

SEQ ID NO: 57 - DNA, 3195 bp, synthetic construct
  misc_feature 1..3195: note = B2E5-48 CAR
  source 1..3195: mol_type = other DNA
  CDS 1..3195
atgctgctgctggtgaccagcctgctgctgtgcgagctgccccaccccgcctttctgctgatccccgacatccagcaaattgttctcacccagtctccagcactcatgtctgcatctccaggggagagggtcaccttgacctgcagtgccagctcaagtgtaggttacatgtactggtaccagcagaagccaggaagctcccccaaaccctggatttatgtcacatccaacctggcttctggagtccctgctcgcttcagtggcagtgggtctgggacctcttactctctcacaatcagcagcatggaggctgaagatgctgccacttattactgccagcagtggagtagtaacccacctacgttcggtgctgggaccaagctggagctgaaacgaactggcagcacctccggcagcggcaagcctggcagcggcgagggcagcaccaagggccaggtccaactccagcagcctggggctgaactggtgaagcctggggcttcagtgaagttgtcctgcaaggcttctggctacaccttcaccaactactggatgcactgggtgaagctgaggcctggacaaggctttgagtggattggagagattaatcctaccaatggtggtactgactacaatgagaagttcaagagaaaggccacactgactgtagacaaatcctccagcacagcctacatgcaactcagcagcctgacatctgaggactctgcggtctattactgcacaatatatactacggctcttgactactggggccaaggcaccactctcacagtctcctcagagcccaaatcttctgacaaaactcacacatctccaccgtgcccagcccccgagttcctgggcggacccagcgtgttcctgttcccccccaagcccaaggacaccctgatgatcagccggacccccgaggtgacctgcgtggtggtggacgtgagccaggaagatcccgaggtccagttcaattggtacgtggacggcgtggaagtgcacaacgccaagaccaagcccagagaggaacagttcaacagcacctaccgggtggtgtctgtgctgaccgtgctgcaccaggactggctgaacggcaaagaatacaagtgcaaggtgtccaacaagggcctgcccagcagcatcgaaaagaccatcagcaaggccaagggccagcctcgcgagccccaggtgtacaccctgcctccctcccaggaagagatgaccaagaaccaggtgtccctgacctgcctggtgaagggcttctaccccagcgacatcgccgtggagtgggagagcaacggccagcctgagaacaactacaagaccacccctcccgtgctggacagcgacggcagcttcttcctgtacagccggctgaccgtggacaagagccggtggcaggaaggcaacgtctttagctgcagcgtgatgcacgaggccctgcacaaccactacacccagaagagcctgagcctgtccctgggcaagatgttctgggtgctggtggtggtgggcggggtgctggcctgctacagcctgctggtgacagtggccttcatcatcttttgggtgcggagcaagcggagcagaggcggccacagcgactacatgaacatgacccccagacggcctggccccacccggaagcactaccagccctacgccccacccagggactttgccgcctaccggtccggcggagggcgggtgaagttcagcagaagcgccgacgcccctgcctaccagcagggccagaatcagctgtacaacgagctgaacctgggcagaagggaagagtacgacgtcctggataagcggagaggccgggaccctgagatgggcggcaagcctcggcggaagaacccccaggaaggcctgtataacgaactgcagaaagacaagatggccgaggcctacagcgagatcggcatgaagggcgagcggaggcggggcaagggccacgacggcctgtatcagggcctgtccaccgccaccaaggatacctacgacgccctgcacatgcaggccctgcccccaaggctcgagggcggcggagagggcagaggaagtcttctaacatgcggtgacgtggaggagaatcccggccctaggatgcttctcctggtgacaagccttctgctctgtgagttaccacacccagcattcctcctgatcccacgcaaagtgtgtaacggaataggtattggtgaatttaaagactcactctccataaatgctacgaatattaaacacttcaaaaactgcacctccatcagtggcgatctccacatcctgccggtggcatttaggggtgactccttcacacatactcctcctctggatccacaggaactggatattctgaaaaccgtaaaggaaatcacagggtttttgctgattcaggcttggcctgaaaacaggacggacctccatgcctttgagaacctagaaatcatacgcggcaggaccaagcaacatggtcagttttctcttgcagtcgtcagcctgaacataacatccttgggattacgctccctcaaggagataagtgatggagatgtgataatttcaggaaacaaaaatttgtgctatgcaaatacaataaactggaaaaaactgtttgggacctccggtcagaaaaccaaaattataagcaacagaggtgaaaacagctgcaaggccacaggccaggtctgccatgccttgtgctcccccgagggctgctggggcccggagcccagggactgcgtctcttgccggaatgtcagccgaggcagggaatgcgtggacaagtgcaaccttctggagggtgagccaagggagtttgtggagaactctgagtgcatacagtgccacccagagtgcctgcctcaggccatgaacatcacctgcacaggacggggaccagacaactgtatccagtgtgcccactacattgacggcccccactgcgtcaagacctgcccggcaggagtcatgggagaaaacaacaccctggtctggaagtacgcagacgccggccatgtgtgccacctgtgccatccaaactgcacctacggatgcactgggccaggtcttgaaggctgtccaacgaatgggcctaagatcccgtccatcgccactgggatggtgggggccctcctcttgctgctggtggtggccctggggatcggcctcttcatgtga

SEQ ID NO: 58 - protein, 1064 aa, synthetic construct
  REGION 1..1064: note = B2E5-48 CAR
  SITE 1..25: note = GM-CSF leader sequence
  SITE 26..131: note = Variable Region of Light Chain (B2E5-48)
  SITE 134..151: note = 18aa Linke
  SITE 152..267: note = Variable Region of Heavy Chain (B2E5-48)
  SITE 268..282: note = FC
  SITE 283..392: note = CH2
  SITE 393..499: note = CH3
  SITE 500..527: note = CD28TM
  SITE 528..568: note = CD28IC
  SITE 569..571: note = GGG
  SITE 572..688: note = CD3z
  SITE 689..707: note = T2A
  SITE 708..1064: note = tEGFR
MLLLVTSLLLCELPHPAFLLIPDIQQIVLTQSPALMSASPGERVTLTCSASSSVGYMYWYQQKPGSSPKPWIYVTSNLASGVPARFSGSGSGTSYSLTISSMEAEDAATYYCQQWSSNPPTFGAGTKLELKRTGSTSGSGKPGSGEGSTKGQVQLQQPGAELVKPGASVKLSCKASGYTFTNYWMHWVKLRPGQGFEWIGEINPTNGGTDYNEKFKRKATLTVDKSSSTAYMQLSSLTSEDSAVYYCTIYTTALDYWGQGTTLTVSSEPKSSDKTHTSPPCPAPEFLGGPSVFLFPPKPKDTLMISRTPEVTCVVVDVSQEDPEVQFNWYVDGVEVHNAKTKPREEQFNSTYRVVSVLTVLHQDWLNGKEYKCKVSNKGLPSSIEKTISKAKGQPREPQVYTLPPSQEEMTKNQVSLTCLVKGFYPSDIAVEWESNGQPENNYKTTPPVLDSDGSFFLYSRLTVDKSRWQEGNVFSCSVMHEALHNHYTQKSLSLSLGKMFWVLVVVGGVLACYSLLVTVAFIIFWVRSKRSRGGHSDYMNMTPRRPGPTRKHYQPYAPPRDFAAYRSGGGRVKFSRSADAPAYQQGQNQLYNELNLGRREEYDVLDKRRGRDPEMGGKPRRKNPQEGLYNELQKDKMAEAYSEIGMKGERRRGKGHDGLYQGLSTATKDTYDALHMQALPPRLEGGGEGRGSLLTCGDVEENPGPRMLLLVTSLLLCELPHPAFLLIPRKVCNGIGIGEFKDSLSINATNIKHFKNCTSISGDLHILPVAFRGDSFTHTPPLDPQELDILKTVKEITGFLLIQAWPENRTDLHAFENLEIIRGRTKQHGQFSLAVVSLNITSLGLRSLKEISDGDVIISGNKNLCYANTINWKKLFGTSGQKTKIISNRGENSCKATGQVCHALCSPEGCWGPEPRDCVSCRNVSRGRECVDKCNLLEGEPREFVENSECIQCHPECLPQAMNITCTGRGPDNCIQCAHYIDGPHCVKTCPAGVMGENNTLVWKYADAGHVCHLCHPNCTYGCTGPGLEGCPTNGPKIPSIATGMVGALLLLLVVALGIGLFM

SEQ ID NO: 59 - protein, 15 aa, synthetic construct
  REGION 1..15: note = Hinge region:15aa
EPKSSDKTHTSPPCP

SEQ ID NO: 60 - protein, 30 aa, synthetic construct
  REGION 1..30: note = Hinge region:30aa
EPKSSDKTHTSPPCPAPEFLGGPSVFLFPP

SEQ ID NO: 61 - protein, 60 aa, synthetic construct
  REGION 1..60: note = Hinge region:60aa
EPKSSDKTHTSPPCPAPEFLGGPSVFLFPPKPKDTLMISRTPEVTCVVVDVSQEDPEVQF

SEQ ID NO: 62 - protein, 125 aa, synthetic construct
  REGION 1..125: note = Hinge region:125aa
EPKSSDKTHTSPPCPAPEFLGGPSVFLFPPKPKDTLMISRTPEVTCVVVDVSQEDPEVQFNWYVDGVEVHNAKTKPREEQFNSTYRVVSVLTVLHQDWLNGKEYKCKVSNKGLPSSIEKTISKAK

SEQ ID NO: 63 - protein, 232 aa, synthetic construct
  REGION 1..232: note = Hinge region:232aa
EPKSSDKTHTSPPCPAPEFLGGPSVFLFPPKPKDTLMISRTPEVTCVVVDVSQEDPEVQFNWYVDGVEVHNAKTKPREEQFNSTYRVVSVLTVLHQDWLNGKEYKCKVSNKGLPSSIEKTISKAKGQPREPQVYTLPPSQEEMTKNQVSLTCLVKGFYPSDIAVEWESNGQPENNYKTTPPVLDSDGSFFLYSRLTVDKSRWQEGNVFSCSVMHEALHNHYTQKSLSLSLGK

SEQ ID NO: 64 - protein, 42 aa, synthetic construct
  REGION 1..42: note = 4-1BB IC
KRGRKKLLYIFKQPFMRPVQTTQEEDGCSCRFPEEEEGGCEL

SEQ ID NO: 65 - protein, 61 aa, synthetic construct
  REGION 1..61: note = CD79A IC
RKRWQNEKLGLDAGDEYEDENLYEGLNLDDCSMYEDISRGLQGTYQDVGSLNIGDVQLEKP

SEQ ID NO: 66 - protein, 62 aa, synthetic construct
  REGION 1..62: note = CD40 IC
KKVAKKPTNKAPHPKQEPQEINFPDDLPGSNTAAPVQETLHGCQPVTQEDGKESRISVQERQ